European Patent Application EP 4 806 465 A2, published September 16, 2026. Title: C-TYPE NATRIURETIC PEPTIDES AND METHODS THEREOF IN TREATING ACUTE LUNG INJURY. Applicant: Pharmain Corporation. Application EP. The sequence listing filed with the application follows.

SEQUENCE LISTING (30 sequences)

SEQ ID NO: 1 - protein, 39 aa, synthetic construct
  REGION 1..39: note = Synthetic
PGQEHPNARKYKGANKKGLSKGCFGLKLDRIGSMSGLGC

SEQ ID NO: 2 - protein, 23 aa, synthetic construct
  REGION 1..23: note = Synthetic
  SITE 1: note = Wherein X at position 1 is defined as the entirety of either (aliphatic)a-(X)- or (polymer)a-(Y)- as defined in the specification
XGLSKGCFGLKLDRIGSMSGLGC

SEQ ID NO: 3 - protein, 24 aa, synthetic construct
  REGION 1..24: note = Synthetic
  SITE 1: note = Wherein X at position 1 is defined as the entirety of either (aliphatic)a-(X)- or (polymer)a-(Y)- as defined in the specification
  SITE 11: note = Wherein X at position 11 is defined as the entirety of either (aliphatic)a-(X)- or (polymer)a-(Y)- as defined in the specification
  VARIANT 12: note = Xaa can be any naturally occurring amino acid
XGLSKGCFGLKXLDRIGSMSGLGC

SEQ ID NO: 4 - protein, 23 aa, synthetic construct
  REGION 1..23: note = Synthetic
  SITE 11: note = Wherein X at position 11 is defined as the entirety of either (aliphatic)a-(X)- or (polymer)a-(Y)- as defined in the specification
GLSKGCFGLKXLDRIGSMSGLGC

SEQ ID NO: 5 - protein, 29 aa, synthetic construct
  REGION 1..29: note = Synthetic
KKKKGGGGLSKGCFGLKLDRIGSMSGLGC

SEQ ID NO: 6 - protein, 29 aa, synthetic construct
  REGION 1..29: note = Synthetic
KKKKGGGGLSKGCFGLKLDRIGSMSGLGC

SEQ ID NO: 7 - protein, 29 aa, synthetic construct
  REGION 1..29: note = Synthetic
KKKKGGGGLSKGCFGLKLDRIGSMSGLGC

SEQ ID NO: 8 - protein, 29 aa, synthetic construct
  REGION 1..29: note = Synthetic
KKKKGGGGLSKGCFGLKLDRIGSMSGLGC

SEQ ID NO: 9 - protein, 29 aa, synthetic construct
  REGION 1..29: note = Synthetic
KKKKGGGGLSKGCFGLKLDRIGSMSGLGC

SEQ ID NO: 10 - protein, 22 aa, synthetic construct
  REGION 1..22: note = Synthetic
GLSKGCFGLKLDRIGSMSGLGC

SEQ ID NO: 11 - protein, 18 aa, synthetic construct
  REGION 1..18: note = Synthetic
  SITE 1: note = Wherein X at position 1 is defined as the entirety of either (aliphatic)a-(X)- or (polymer)a-(Y)- as defined in the specification
  VARIANT 13: note = Wherein X at position 13 is defined as a natural or unnatural amino acid as defined in the specification
XCFGLKLDRIGSXSGLGC

SEQ ID NO: 12 - protein, 18 aa, synthetic construct
  REGION 1..18: note = Synthetic
  SITE 1: note = Wherein X at position 1 is defined as (aliphatic)a-(X)- as defined in the specification
  VARIANT 13: note = Wherein X at position 13 is defined as a natural or unnatural aminio acid as defined in the specification
XCFGLKLDRIGSXSGLGC

SEQ ID NO: 13 - protein, 18 aa, synthetic construct
  REGION 1..18: note = Synthetic
  SITE 1: note = Wherein X at position 1 is defined as (aliphatic)a-((gammaE)0-2-Gly)- as defined in the specification
  SITE 13: note = Wherein X at position 13 is defined as homoglutamine as defined in the specification
XCFGLKLDRIGSXSGLGC

SEQ ID NO: 14 - protein, 18 aa, synthetic construct
  REGION 1..18: note = Synthetic
  SITE 1: note = Wherein X at position 1 is defined as (aliphatic)a-(gammaE-Gly)- as defined in the specification
  SITE 13: note = Wherein X at position 13 is defined as homoglutamine as defined in the specification
XCFGLKLDRIGSXSGLGC

SEQ ID NO: 15 - protein, 18 aa, synthetic construct
  REGION 1..18: note = Synthetic
  SITE 1: note = Wherein X at position 1 is defined as (aliphatic)a-(gammaE)- as defined in the specification
  SITE 13: note = Wherein X at position 13 is defined as homoglutamine as defined in the specification
XCFGLKLDRIGSXSGLGC

SEQ ID NO: 16 - protein, 18 aa, synthetic construct
  REGION 1..18: note = Synthetic
  SITE 1: note = Wherein X at position 1 is defined as (aliphatic)a-2-[2-(2-aminoethoxy)ethoxy]acetic acid-2-[2-(2-aminoethoxy)ethoxy]acetic acid- as defined in the specification
  SITE 13: note = Wherein X at position 13 is defined as homoglutamine as defined in the specification
XCFGLKLDRIGSXSGLGC

SEQ ID NO: 17 - protein, 18 aa, synthetic construct
  REGION 1..18: note = Synthetic
  SITE 1: note = Wherein X at position 1 is defined as (aliphatic)a-gammaE-2-[2-(2-aminoethoxy)ethoxy]acetic acid-2-[2-(2-aminoethoxy)ethoxy]acetic acid- as defined in the specification
  SITE 13: note = Wherein X at position 13 is defined as homoglutamine as defined in the specification
XCFGLKLDRIGSXSGLGC

SEQ ID NO: 18 - protein, 18 aa, synthetic construct
  REGION 1..18: note = Synthetic
  SITE 1: note = Wherein X at position 1 is defined as (aliphatic)a-2-[2-(2-aminoethoxy)ethoxy]acetic acid-2-[2-(2-aminoethoxy)ethoxy]acetic acid-Gly- as defined in the specification
  SITE 13: note = Wherein X at position 13 is defined as homoglutamine as defined in the specification
XCFGLKLDRIGSXSGLGC

SEQ ID NO: 19 - protein, 18 aa, synthetic construct
  REGION 1..18: note = Synthetic
  SITE 1: note = Wherein X at position 1 is defined as (aliphatic)a-gammaE-2-[2-(2-aminoethoxy)ethoxy]acetic acid-2-[2-(2-aminoethoxy)ethoxy]acetic acid-Gly- as defined in the specification
  SITE 13: note = Wherein X at position 13 is defined as homoglutamine as defined in the specification
XCFGLKLDRIGSXSGLGC

SEQ ID NO: 20 - protein, 18 aa, synthetic construct
  REGION 1..18: note = Synthetic
  SITE 1: note = Wherein X at position 1 is defined as HOC(=O)(CH2)16C(=O)-gammaE-2-[2-(2-aminoethoxy)ethoxy]acetic acid-2-[2-(2-aminoethoxy)ethoxy]acetic acid-Gly- as defined in the specification
  SITE 13: note = Wherein X at position 13 is defined as homoglutamine as defined in the specification
XCFGLKLDRIGSXSGLGC

SEQ ID NO: 21 - protein, 18 aa, synthetic construct
  REGION 1..18: note = Synthetic
  SITE 1: note = Wherein X at position 1 is defined as HOC(=O)(CH2)16C(=O)-2-[2-(2-aminoethoxy)ethoxy]acetic acid-2-[2-(2-aminoethoxy)ethoxy]acetic acid-Gly- as defined in the specification
  SITE 13: note = Wherein X at position 13 is defined as homoglutamine as defined in the specification
XCFGLKLDRIGSXSGLGC

SEQ ID NO: 22 - protein, 8 aa, synthetic construct
  REGION 1..8: note = Synthetic
  SITE 1: note = Wherein X at position 1 is defined as CH3(CH2)14C(=O)- as defined in the specification
XKKKKGGG

SEQ ID NO: 23 - protein, 8 aa, synthetic construct
  REGION 1..8: note = Synthetic
  SITE 1: note = Wherein X at position 1 is defined as CH3(CH2)16C(=O)- as defined in the specification
XKKKKGGG

SEQ ID NO: 24 - protein, 8 aa, synthetic construct
  REGION 1..8: note = Synthetic
  SITE 1: note = Wherein X at position 1 is defined as CH3(CH2)18C(=O)- as defined in the specification
XKKKKGGG

SEQ ID NO: 25 - protein, 8 aa, synthetic construct
  REGION 1..8: note = Synthetic
  SITE 1: note = Wherein X at position 1 is defined as CH3(CH2)20C(=O)- as defined in the specification
XKKKKGGG

SEQ ID NO: 26 - protein, 8 aa, synthetic construct
  REGION 1..8: note = Synthetic
  SITE 1: note = Wherein X at position 1 is defined as CH3(CH2)22C(=O)- as defined in the specification
XKKKKGGG

SEQ ID NO: 27 - protein, 18 aa, synthetic construct
  REGION 1..18: note = Synthetic
  SITE 1: note = Wherein X at position 1 is defined as (polymer)a-(Y)- as defined in the specification
  VARIANT 13: note = Wherein X at position 13 is defined as a natural or unnatural amino acid as defined in the specification
XCFGLKLDRIGSXSGLGC

SEQ ID NO: 28 - protein, 36 aa, synthetic construct
  REGION 1..36: note = Synthetic
  SITE 1: note = Wherein X at position 1 is defined as CH3(CH2)16C(=O)- as defined in the specification
XKKKKGGGSLRRSSCFGGRMDRIGAQSGLGCNSFRY

SEQ ID NO: 29 - protein, 40 aa, synthetic construct
  REGION 1..40: note = Synthetic
  SITE 1: note = Wherein X at position 1 is defined as CH3(CH2)16C(=O)- as defined in the specification
XKKKKGGGSPKMVQGSGCFGRKMDRISSSSGLGCKVLRRH

SEQ ID NO: 30 - protein, 18 aa, synthetic construct
  REGION 1..18: note = Synthetic
  SITE 1: note = Wherein X at position 1 is defined as (aliphatic)a-(X)- as defined in the specification
  VARIANT 13: note = Wherein X at position 13 is defined as a natural or unnatural amino acid, but not methionine as defined in the specification
XCFGLKLDRIGSXSGLGC